European Patent Specification EP 3 273 944 B1, published November 20, 2024. Title: COMPOSITIONS AND METHODS FOR DELIVERY OF BIOMACROMOLECULE AGENTS. Applicant: THE REGENTS OF THE UNIVERSITY OF MICHIGAN. The sequence listing filed with the application follows.

SEQUENCE LISTING (340 sequences)

SEQ ID NO: 1 - protein, 22 aa, Artificial sequence
  synthetic
PVLDLFRELLNELLEZLKQKLK

SEQ ID NO: 2 - protein, 23 aa, Artificial sequence
  synthetic
GVLDLFRELLNELLEALKQKLKK

SEQ ID NO: 3 - protein, 22 aa, Artificial sequence
  synthetic
PVLDLFRELLNELLEWLKQKLK

SEQ ID NO: 4 - protein, 22 aa, Artificial sequence
  synthetic
PVLDLFRELLNELLEALKQKLK

SEQ ID NO: 5 - protein, 23 aa, Artificial sequence
  synthetic
PVLDLFRELLNELLEALKQKLKK

SEQ ID NO: 6 - protein, 22 aa, Artificial sequence
  synthetic
  misc_feature: Xaa = Aib
  misc_feature (13)..(13): Xaa can be any naturally occurring amino acid
PVLDLFRELLNEXLEALKQKLK

SEQ ID NO: 7 - protein, 22 aa, Artificial sequence
  synthetic
PVLDLFKELLNELLEALKQKLK

SEQ ID NO: 8 - protein, 22 aa, Artificial sequence
  synthetic
PVLDLFRELLNEGLEALKQKLK

SEQ ID NO: 9 - protein, 22 aa, Artificial sequence
  synthetic
PVLDLFRELGNELLEALKQKLK

SEQ ID NO: 10 - protein, 22 aa, Artificial sequence
  synthetic
PVLDLFRELLNELLEAZKQKLK

SEQ ID NO: 11 - protein, 22 aa, Artificial sequence
  synthetic
PVLDLFKELLQELLEALKQKLK

SEQ ID NO: 12 - protein, 22 aa, Artificial sequence
  synthetic
PVLDLFRELLNELLEAGKQKLK

SEQ ID NO: 13 - protein, 22 aa, Artificial sequence
  synthetic
GVLDLFRELLNEGLEALKQKLK

SEQ ID NO: 14 - protein, 22 aa, Artificial sequence
  synthetic
  misc_feature: Xaa = Orn
  misc_feature (18)..(18): Xaa can be any naturally occurring amino acid
  misc_feature (20)..(20): Xaa can be any naturally occurring amino acid
  misc_feature (22)..(22): Xaa can be any naturally occurring amino acid
PVLDLFRELLNELLEALXQXLX

SEQ ID NO: 15 - protein, 22 aa, Artificial sequence
  synthetic
PVLDLFRELWNELLEALKQKLK

SEQ ID NO: 16 - protein, 22 aa, Artificial sequence
  synthetic
PVLDLLRELLNELLEALKQKLK

SEQ ID NO: 17 - protein, 22 aa, Artificial sequence
  synthetic
PVLELFKELLQELLEALKQKLK

SEQ ID NO: 18 - protein, 22 aa, Artificial sequence
  synthetic
GVLDLFRELLNELLEALKQKLK

SEQ ID NO: 19 - protein, 22 aa, Artificial sequence
  synthetic
PVLDLFRELLNEGLEALKQKLK

SEQ ID NO: 20 - protein, 22 aa, Artificial sequence
  synthetic
PVLDLFREGLNELLEALKQKLK

SEQ ID NO: 21 - protein, 22 aa, Artificial sequence
  synthetic
PVLDLFRELLNELLEALKQKLK

SEQ ID NO: 22 - protein, 22 aa, Artificial sequence
  synthetic
PVLDLFRELLNELLEGLKQKLK

SEQ ID NO: 23 - protein, 22 aa, Artificial sequence
  synthetic
PLLELFKELLQELLEALKQKLK

SEQ ID NO: 24 - protein, 22 aa, Artificial sequence
  synthetic
PVLDLFRELLNELLEALQKKLK

SEQ ID NO: 25 - protein, 22 aa, Artificial sequence
  synthetic
  misc_feature: Xaa = Aib
  misc_feature (13)..(13): Xaa can be any naturally occurring amino acid
PVLDFFRELLNEXLEALKQKLK

SEQ ID NO: 26 - protein, 22 aa, Artificial sequence
  synthetic
PVLDLFRELLNELLELLKQKLK

SEQ ID NO: 27 - protein, 22 aa, Artificial sequence
  synthetic
PVLDLFRELLNELZEALKQKLK

SEQ ID NO: 28 - protein, 22 aa, Artificial sequence
  synthetic
PVLDLFRELLNELWEALKQKLK

SEQ ID NO: 29 - protein, 22 aa, Artificial sequence
  synthetic
AVLDLFRELLNELLEALKQKLK

SEQ ID NO: 30 - protein, 22 aa, Artificial sequence
  synthetic
PVLDLPRELLNELLEALKQKLK

SEQ ID NO: 31 - protein, 22 aa, Artificial sequence
  synthetic
  misc_feature: Xaa = Aib
  misc_feature (13)..(13): Xaa can be any naturally occurring amino acid
PVLDLFLELLNEXLEALKQKLK

SEQ ID NO: 32 - protein, 22 aa, Artificial sequence
  synthetic
  misc_feature: Xaa = Aib
  misc_feature (1)..(1): Xaa can be any naturally occurring amino acid
XVLDLFRELLNELLEALKQKLK

SEQ ID NO: 33 - protein, 22 aa, Artificial sequence
  synthetic
PVLDLFREKLNELLEALKQKLK

SEQ ID NO: 34 - protein, 22 aa, Artificial sequence
  synthetic
PVLDZFRELLNELLEALKQKLK

SEQ ID NO: 35 - protein, 22 aa, Artificial sequence
  synthetic
PVLDWFRELLNELLEALKQKLK

SEQ ID NO: 36 - protein, 22 aa, Artificial sequence
  synthetic
PLLELLKELLQELLEALKQKLK

SEQ ID NO: 37 - protein, 22 aa, Artificial sequence
  synthetic
PVLDLFREWLNELLEALKQKLK

SEQ ID NO: 38 - protein, 22 aa, Artificial sequence
  synthetic
  misc_feature: Xaa = Aib
  misc_feature (13)..(13): Xaa can be any naturally occurring amino acid
PVLDLFRELLNEXLEAWKQKLK

SEQ ID NO: 39 - protein, 22 aa, Artificial sequence
  synthetic
PVLDLFRELLEELLKALKKKLK

SEQ ID NO: 40 - protein, 22 aa, Artificial sequence
  synthetic
PVLDLFNELLRELLEALQKKLK

SEQ ID NO: 41 - protein, 22 aa, Artificial sequence
  synthetic
  misc_feature: Xaa = Aib
  misc_feature (13)..(13): Xaa can be any naturally occurring amino acid
PVLDLWRELLNEXLEALKQKLK

SEQ ID NO: 42 - protein, 22 aa, Artificial sequence
  synthetic
  misc_feature: Xaa = Aib
  misc_feature (13)..(13): Xaa can be any naturally occurring amino acid
PVLDEFREKLNEXWEALKQKLK

SEQ ID NO: 43 - protein, 22 aa, Artificial sequence
  synthetic
  misc_feature: Xaa = Aib
  misc_feature (13)..(13): Xaa can be any naturally occurring amino acid
PVLDEFREKLWEXLEALKQKLK

SEQ ID NO: 44 - protein, 22 aa, Artificial sequence
  synthetic
  misc_feature: Xaa = Aib
  misc_feature (13)..(13): Xaa can be any naturally occurring amino acid
PVLDEFREKLNEXLEALKQKLK

SEQ ID NO: 45 - protein, 22 aa, Artificial sequence
  synthetic
  misc_feature: Xaa = Aib
  misc_feature (13)..(13): Xaa can be any naturally occurring amino acid
PVLDEFREKLNEXLEALKQKLK

SEQ ID NO: 46 - protein, 22 aa, Artificial sequence
  synthetic
  misc_feature: Xaa = Aib
  misc_feature (13)..(13): Xaa can be any naturally occurring amino acid
PVLDLFREKLNEXLEALKQKLK

SEQ ID NO: 47 - protein, 21 aa, Artificial sequence
  synthetic
VLDLFRELLNEGLEALKQKLK

SEQ ID NO: 48 - protein, 22 aa, Artificial sequence
  synthetic
PVLDLFRELLNELLEALKQKLK

SEQ ID NO: 49 - protein, 22 aa, Artificial sequence
  synthetic
PVLDLFRNLLEKLLEALEQKLK

SEQ ID NO: 50 - protein, 22 aa, Artificial sequence
  synthetic
  misc_feature: Xaa = Aib
  misc_feature (13)..(13): Xaa can be any naturally occurring amino acid
PVLDLFRELLWEXLEALKQKLK

SEQ ID NO: 51 - protein, 22 aa, Artificial sequence
  synthetic
  misc_feature: Xaa = Aib
  misc_feature (13)..(13): Xaa can be any naturally occurring amino acid
PVLDLFWELLNEXLEALKQKLK

SEQ ID NO: 52 - protein, 22 aa, Artificial sequence
  synthetic
  misc_feature: Xaa = Aib
  misc_feature (13)..(13): Xaa can be any naturally occurring amino acid
PVWDEFREKLNEXLEALKQKLK

SEQ ID NO: 53 - protein, 22 aa, Artificial sequence
  synthetic
VVLDLFRELLNELLEALKQKLK

SEQ ID NO: 54 - protein, 22 aa, Artificial sequence
  synthetic
PVLDLFRELLNEWLEALKQKLK

SEQ ID NO: 55 - protein, 19 aa, Artificial sequence
  synthetic
PLFRELLNELLEALKQKLK

SEQ ID NO: 56 - protein, 22 aa, Artificial sequence
  synthetic
PVLDLFRELLNELLEALKQKKK

SEQ ID NO: 57 - protein, 22 aa, Artificial sequence
  synthetic
PVLDLFRNLLEELLKALEQKLK

SEQ ID NO: 58 - protein, 21 aa, Artificial sequence
  synthetic
  misc_feature: Xaa = Aib
  misc_feature (13)..(13): Xaa can be any naturally occurring amino acid
PVLDEFREKLNEXLEALKQKL

SEQ ID NO: 59 - protein, 22 aa, Artificial sequence
  synthetic
LVLDLFRELLNELLEALKQKLK

SEQ ID NO: 60 - protein, 19 aa, Artificial sequence
  synthetic
PVLDLFRELLNELLEALKQ

SEQ ID NO: 61 - protein, 22 aa, Artificial sequence
  synthetic
  misc_feature: Xaa = Aib
  misc_feature (13)..(13): Xaa can be any naturally occurring amino acid
PVLDEFRWKLNEXLEALKQKLK

SEQ ID NO: 62 - protein, 22 aa, Artificial sequence
  synthetic
  misc_feature: Xaa = Aib
  misc_feature (13)..(13): Xaa can be any naturally occurring amino acid
PVLDEWREKLNEXLEALKQKLK

SEQ ID NO: 63 - protein, 22 aa, Artificial sequence
  synthetic
  misc_feature: Xaa = Aib
  misc_feature (13)..(13): Xaa can be any naturally occurring amino acid
PVLDFFREKLNEXLEALKQKLK

SEQ ID NO: 64 - protein, 22 aa, Artificial sequence
  synthetic
  misc_feature: Xaa = Aib
  misc_feature (13)..(13): Xaa can be any naturally occurring amino acid
PWLDEFREKLNEXLEALKQKLK

SEQ ID NO: 65 - protein, 21 aa, Artificial sequence
  synthetic
  misc_feature: Xaa = Aib
  misc_feature (12)..(12): Xaa can be any naturally occurring amino acid
VLDEFREKLNEXLEALKQKLK

SEQ ID NO: 66 - protein, 22 aa, Artificial sequence
  synthetic
PVLDLFRNLLEELLEALQKKLK

SEQ ID NO: 67 - protein, 21 aa, Artificial sequence
  synthetic
VLDLFRELLNELLEALKQKLK

SEQ ID NO: 68 - protein, 22 aa, Artificial sequence
  synthetic
  misc_feature: Xaa = Aib
  misc_feature (13)..(13): Xaa can be any naturally occurring amino acid
PVLDEFRELLKEXLEALKQKLK

SEQ ID NO: 69 - protein, 22 aa, Artificial sequence
  synthetic
  misc_feature: Xaa = Aib
  misc_feature (13)..(13): Xaa can be any naturally occurring amino acid
PVLDEFRKKLNEXLEALKQKLK

SEQ ID NO: 70 - protein, 22 aa, Artificial sequence
  synthetic
  misc_feature: Xaa = Aib
  misc_feature (13)..(13): Xaa can be any naturally occurring amino acid
PVLDEFRELLYEXLEALKQKLK

SEQ ID NO: 71 - protein, 22 aa, Artificial sequence
  synthetic
  misc_feature: Xaa = Aib
  misc_feature (14)..(14): Xaa can be any naturally occurring amino acid
PVLDEFREKLNELXEALKQKLK

SEQ ID NO: 72 - protein, 22 aa, Artificial sequence
  synthetic
  misc_feature: Xaa = Aib
  misc_feature (13)..(13): Xaa can be any naturally occurring amino acid
PVLDLFRELLNEXLWALKQKLK

SEQ ID NO: 73 - protein, 22 aa, Artificial sequence
  synthetic
  misc_feature: Xaa = Aib
  misc_feature (13)..(13): Xaa can be any naturally occurring amino acid
PVLDEFWEKLNEXLEALKQKLK

SEQ ID NO: 74 - protein, 22 aa, Artificial sequence
  synthetic
  misc_feature: Xaa = Aib
  misc_feature (13)..(13): Xaa can be any naturally occurring amino acid
PVLDKFREKLNEXLEALKQKLK

SEQ ID NO: 75 - protein, 22 aa, Artificial sequence
  synthetic
PVLDEFREKLNEELEALKQKLK

SEQ ID NO: 76 - protein, 22 aa, Artificial sequence
  synthetic
  misc_feature: Xaa = Aib
  misc_feature (13)..(13): Xaa can be any naturally occurring amino acid
PVLDEFRELLFEXLEALKQKLK

SEQ ID NO: 77 - protein, 22 aa, Artificial sequence
  synthetic
  misc_feature: Xaa = Aib
  misc_feature (13)..(13): Xaa can be any naturally occurring amino acid
PVLDEFREKLNKXLEALKQKLK

SEQ ID NO: 78 - protein, 22 aa, Artificial sequence
  synthetic
  misc_feature (13)..(13): Xaa can be any naturally occurring amino acid
PVLDEFRDKLNEXLEALKQKLK

SEQ ID NO: 79 - protein, 22 aa, Artificial sequence
  synthetic
PVLDEFRELLNELLEALKQKLK

SEQ ID NO: 80 - protein, 22 aa, Artificial sequence
  synthetic
PVLDLFERLLNELLEALQKKLK

SEQ ID NO: 81 - protein, 22 aa, Artificial sequence
  synthetic
  misc_feature: Xaa = Aib
  misc_feature (13)..(13): Xaa can be any naturally occurring amino acid
PVLDEFREKLNWXLEALKQKLK

SEQ ID NO: 82 - protein, 20 aa, Artificial sequence
  synthetic
  misc_feature: Xaa = Aib
  misc_feature (11)..(11): Xaa can be any naturally occurring amino acid
LDEFREKLNEXLEALKQKLK

SEQ ID NO: 83 - protein, 22 aa, Artificial sequence
  synthetic
  misc_feature: Xaa = Aib
  misc_feature (13)..(13): Xaa can be any naturally occurring amino acid
PVLDEFREKLNEXLEALWQKLK

SEQ ID NO: 84 - protein, 22 aa, Artificial sequence
  synthetic
PVLDEFREKLNELLEALKQKLK

SEQ ID NO: 85 - protein, 21 aa, Artificial sequence
  synthetic
PLDLFRELLNELLEALKQKLK

SEQ ID NO: 86 - protein, 22 aa, Artificial sequence
  synthetic
PVLELFERLLDELLNALQKKLK

SEQ ID NO: 87 - protein, 22 aa, Artificial sequence
  synthetic
PLLELLKELLQELLEALKQKLK

SEQ ID NO: 88 - protein, 22 aa, Artificial sequence
  synthetic
  misc_feature: Xaa = Aib
  misc_feature (13)..(13): Xaa can be any naturally occurring amino acid
PVLDKFRELLNEXLEALKQKLK

SEQ ID NO: 89 - protein, 22 aa, Artificial sequence
  synthetic
  misc_feature: Xaa = Aib
  misc_feature (13)..(13): Xaa can be any naturally occurring amino acid
PVLDEFREKLNEXLWALKQKLK

SEQ ID NO: 90 - protein, 19 aa, Artificial sequence
  synthetic
  misc_feature: Xaa = Aib
  misc_feature (10)..(10): Xaa can be any naturally occurring amino acid
DEFREKLNEXLEALKQKLK

SEQ ID NO: 91 - protein, 22 aa, Artificial sequence
  synthetic
  misc_feature: Xaa = Aib
  misc_feature (13)..(13): Xaa can be any naturally occurring amino acid
PVLDEFRELLNEXLEALKQKLK

SEQ ID NO: 92 - protein, 22 aa, Artificial sequence
  synthetic
  misc_feature: Xaa = Aib
  misc_feature (13)..(13): Xaa can be any naturally occurring amino acid
PVLDEFRELYNEXLEALKQKLK

SEQ ID NO: 93 - protein, 22 aa, Artificial sequence
  synthetic
  misc_feature: Xaa = Aib
  misc_feature (13)..(13): Xaa can be any naturally occurring amino acid
PVLDEFREKLNEXLKALKQKLK

SEQ ID NO: 94 - protein, 22 aa, Artificial sequence
  synthetic
PVLDEFREKLNEALEALKQKLK

SEQ ID NO: 95 - protein, 22 aa, Artificial sequence
  synthetic
  misc_feature: Xaa = Aib
  misc_feature (13)..(13): Xaa can be any naturally occurring amino acid
PVLDLFRELLNLXLEALKQKLK

SEQ ID NO: 96 - protein, 22 aa, Artificial sequence
  synthetic
  misc_feature: Xaa = Aib
  misc_feature (13)..(13): Xaa can be any naturally occurring amino acid
PVLDLFRELLNEXLEALKQKLK

SEQ ID NO: 97 - protein, 15 aa, Artificial sequence
  synthetic
PVLDLFRELLNELLE

SEQ ID NO: 98 - protein, 22 aa, Artificial sequence
  synthetic
PVLDLFRELLNEELEALKQKLK

SEQ ID NO: 99 - protein, 22 aa, Artificial sequence
  synthetic
KLKQKLAELLENLLERFLDLVP

SEQ ID NO: 100 - protein, 22 aa, Artificial sequence
  synthetic
PVLDLFRELLNELLEALKQKLK

SEQ ID NO: 101 - protein, 22 aa, Artificial sequence
  synthetic
  misc_feature: Xaa = Aib
  misc_feature (13)..(13): Xaa can be any naturally occurring amino acid
PVLDLFRELLNWXLEALKQKLK

SEQ ID NO: 102 - protein, 22 aa, Artificial sequence
  synthetic
  misc_feature: Xaa = Aib
  misc_feature (13)..(13): Xaa can be any naturally occurring amino acid
PVLDLFRELLNLXLEALKEKLK

SEQ ID NO: 103 - protein, 22 aa, Artificial sequence
  synthetic
PVLDEFRELLNEELEALKQKLK

SEQ ID NO: 104 - protein, 15 aa, Artificial sequence
  synthetic
PLLNELLEALKQKLK

SEQ ID NO: 105 - protein, 22 aa, Artificial sequence
  synthetic
PAADAFREAANEAAEAAKQKAK

SEQ ID NO: 106 - protein, 22 aa, Artificial sequence
  synthetic
PVLDLFREKLNEELEALKQKLK

SEQ ID NO: 107 - protein, 22 aa, Artificial sequence
  synthetic
KLKQKLAELLENLLERFLDLVP

SEQ ID NO: 108 - protein, 22 aa, Artificial sequence
  synthetic
  misc_feature: Xaa = Aib
  misc_feature (13)..(13): Xaa can be any naturally occurring amino acid
PVLDLFRWLLNEXLEALKQKLK

SEQ ID NO: 109 - protein, 22 aa, Artificial sequence
  synthetic
PVLDEFREKLNERLEALKQKLK

SEQ ID NO: 110 - protein, 22 aa, Artificial sequence
  synthetic
  misc_feature: Xaa = Aib
  misc_feature (13)..(14): Xaa can be any naturally occurring amino acid
PVLDEFREKLNEXXEALKQKLK

SEQ ID NO: 111 - protein, 22 aa, Artificial sequence
  synthetic
  misc_feature: Xaa = Aib
  misc_feature (13)..(13): Xaa can be any naturally occurring amino acid
PVLDEFREKLWEXWEALKQKLK

SEQ ID NO: 112 - protein, 22 aa, Artificial sequence
  synthetic
  misc_feature: Xaa = Aib
  misc_feature (13)..(13): Xaa can be any naturally occurring amino acid
PVLDEFREKLNEXSEALKQKLK

SEQ ID NO: 113 - protein, 22 aa, Artificial sequence
  synthetic
PVLDEFREKLNEPLEALKQKLK

SEQ ID NO: 114 - protein, 22 aa, Artificial sequence
  synthetic
  misc_feature: Xaa = Aib
  misc_feature (13)..(13): Xaa can be any naturally occurring amino acid
PVLDEFREKLNEXMEALKQKLK

SEQ ID NO: 115 - protein, 22 aa, Artificial sequence
  synthetic
  misc_feature: Xaa = Aib
  misc_feature (13)..(13): Xaa can be any naturally occurring amino acid
PKLDEFREKLNEXLEALKQKLK

SEQ ID NO: 116 - protein, 22 aa, Artificial sequence
  synthetic
  misc_feature: Xaa = Aib
  misc_feature (13)..(13): Xaa can be any naturally occurring amino acid
PHLDEFREKLNEXLEALKQKLK

SEQ ID NO: 117 - protein, 22 aa, Artificial sequence
  synthetic
  misc_feature: Xaa = Aib
  misc_feature (13)..(13): Xaa can be any naturally occurring amino acid
PELDEFREKLNEXLEALKQKLK

SEQ ID NO: 118 - protein, 22 aa, Artificial sequence
  synthetic
  misc_feature: Xaa = Aib
  misc_feature (13)..(13): Xaa can be any naturally occurring amino acid
PVLDEFREKLNEXLEALEQKLK

SEQ ID NO: 119 - protein, 22 aa, Artificial sequence
  synthetic
  misc_feature: Xaa = Aib
  misc_feature (17)..(17): Xaa can be any naturally occurring amino acid
PVLDEFREKLNEELEAXKQKLK

SEQ ID NO: 120 - protein, 22 aa, Artificial sequence
  synthetic
  misc_feature: Xaa = Aib
  misc_feature (16)..(16): Xaa can be any naturally occurring amino acid
PVLDEFREKLNEELEXLKQKLK

SEQ ID NO: 121 - protein, 22 aa, Artificial sequence
  synthetic
PVLDEFREKLNEELEALWQKLK

SEQ ID NO: 122 - protein, 22 aa, Artificial sequence
  synthetic
PVLDEFREKLNEELEWLKQKLK

SEQ ID NO: 123 - protein, 22 aa, Artificial sequence
  synthetic
QVLDLFRELLNELLEALKQKLK

SEQ ID NO: 124 - protein, 22 aa, Artificial sequence
  synthetic
  misc_feature: Xaa = Orn
  misc_feature (7)..(7): Xaa can be any naturally occurring amino acid
  misc_feature (18)..(18): Xaa can be any naturally occurring amino acid
  misc_feature (20)..(20): Xaa can be any naturally occurring amino acid
  misc_feature (22)..(22): Xaa can be any naturally occurring amino acid
PVLDLFXELLNELLEALXQXLX

SEQ ID NO: 125 - protein, 22 aa, Artificial sequence
  synthetic
NVLDLFRELLNELLEALKQKLK

SEQ ID NO: 126 - protein, 22 aa, Artificial sequence
  synthetic
PVLDLFRELLNELGEALKQKLK

SEQ ID NO: 127 - protein, 22 aa, Artificial sequence
  synthetic
PVLDLFRELLNELLELLKQKLK

SEQ ID NO: 128 - protein, 22 aa, Artificial sequence
  synthetic
PVLDLFRELLNELLEFLKQKLK

SEQ ID NO: 129 - protein, 22 aa, Artificial sequence
  synthetic
PVLELFNDLLRELLEALQKKLK

SEQ ID NO: 130 - protein, 22 aa, Artificial sequence
  synthetic
PVLELFNDLLRELLEALKQKLK

SEQ ID NO: 131 - protein, 22 aa, Artificial sequence
  synthetic
PVLELFKELLNELLDALRQKLK

SEQ ID NO: 132 - protein, 22 aa, Artificial sequence
  synthetic
PVLDLFRELLENLLEALQKKLK

SEQ ID NO: 133 - protein, 22 aa, Artificial sequence
  synthetic
PVLELFERLLEDLLQALNKKLK

SEQ ID NO: 134 - protein, 22 aa, Artificial sequence
  synthetic
  misc_feature: Xaa = Orn
  misc_feature (19)..(19): Xaa can be any naturally occurring amino acid
PVLELFERLLEDLLKALNXKLK

SEQ ID NO: 135 - protein, 22 aa, Artificial sequence
  synthetic
DVLDLFRELLNELLEALKQKLK

SEQ ID NO: 136 - protein, 22 aa, Artificial sequence
  synthetic
PALELFKDLLQELLEALKQKLK

SEQ ID NO: 137 - protein, 22 aa, Artificial sequence
  synthetic
PVLDLFRELLNEGLEAZKQKLK

SEQ ID NO: 138 - protein, 22 aa, Artificial sequence
  synthetic
PVLDLFRELLNEGLEWLKQKLK

SEQ ID NO: 139 - protein, 22 aa, Artificial sequence
  synthetic
PVLDLFRELWNEGLEALKQKLK

SEQ ID NO: 140 - protein, 22 aa, Artificial sequence
  synthetic
  misc_feature: Xaa = Orn
  misc_feature (18)..(18): Xaa can be any naturally occurring amino acid
  misc_feature (20)..(20): Xaa can be any naturally occurring amino acid
  misc_feature (22)..(22): Xaa can be any naturally occurring amino acid
PVLDLFRELLNEGLEALXQXLX

SEQ ID NO: 141 - protein, 22 aa, Artificial sequence
  synthetic
PVLDFFRELLNEGLEALKQKLK

SEQ ID NO: 142 - protein, 22 aa, Artificial sequence
  synthetic
PVLELFRELLNEGLEALKQKLK

SEQ ID NO: 143 - protein, 22 aa, Artificial sequence
  synthetic
PVLDLFRELLNEGLEALKQKLK

SEQ ID NO: 144 - protein, 22 aa, Artificial sequence
  synthetic
PVLELFENLLERLLDALQKKLK

SEQ ID NO: 145 - protein, 22 aa, Artificial sequence
  synthetic
GVLELFENLLERLLDALQKKLK

SEQ ID NO: 146 - protein, 22 aa, Artificial sequence
  synthetic
PVLELFENLLERLLDALQKKLK

SEQ ID NO: 147 - protein, 22 aa, Artificial sequence
  synthetic
PVLELFENLLERLFDALQKKLK

SEQ ID NO: 148 - protein, 22 aa, Artificial sequence
  synthetic
PVLELFENLLERLGDALQKKLK

SEQ ID NO: 149 - protein, 22 aa, Artificial sequence
  synthetic
PVLELFENLWERLLDALQKKLK

SEQ ID NO: 150 - protein, 22 aa, Artificial sequence
  synthetic
PLLELFENLLERLLDALQKKLK

SEQ ID NO: 151 - protein, 22 aa, Artificial sequence
  synthetic
PVLELFENLGERLLDALQKKLK

SEQ ID NO: 152 - protein, 22 aa, Artificial sequence
  synthetic
PVFELFENLLERLLDALQKKLK

SEQ ID NO: 153 - protein, 22 aa, Artificial sequence
  synthetic
AVLELFENLLERLLDALQKKLK

SEQ ID NO: 154 - protein, 22 aa, Artificial sequence
  synthetic
PVLELFENLLERGLDALQKKLK

SEQ ID NO: 155 - protein, 22 aa, Artificial sequence
  synthetic
PVLELFLNLWERLLDALQKKLK

SEQ ID NO: 156 - protein, 22 aa, Artificial sequence
  synthetic
PVLELFLNLLERLLDALQKKLK

SEQ ID NO: 157 - protein, 22 aa, Artificial sequence
  synthetic
PVLEFFENLLERLLDALQKKLK

SEQ ID NO: 158 - protein, 22 aa, Artificial sequence
  synthetic
PVLELFLNLLERLLDWLQKKLK

SEQ ID NO: 159 - protein, 22 aa, Artificial sequence
  synthetic
PVLDLFENLLERLLDALQKKLK

SEQ ID NO: 160 - protein, 22 aa, Artificial sequence
  synthetic
PVLELFENLLERLLDWLQKKLK

SEQ ID NO: 161 - protein, 22 aa, Artificial sequence
  synthetic
PVLELFENLLERLLEALQKKLK

SEQ ID NO: 162 - protein, 22 aa, Artificial sequence
  synthetic
PVLELFENWLERLLDALQKKLK

SEQ ID NO: 163 - protein, 22 aa, Artificial sequence
  synthetic
PVLELFENLLERLWDALQKKLK

SEQ ID NO: 164 - protein, 22 aa, Artificial sequence
  synthetic
PVLELFENLLERLLDAWQKKLK

SEQ ID NO: 165 - protein, 22 aa, Artificial sequence
  synthetic
PVLELFENLLERLLDLLQKKLK

SEQ ID NO: 166 - protein, 22 aa, Artificial sequence
  synthetic
PVLELFLNLLEKLLDALQKKLK

SEQ ID NO: 167 - protein, 22 aa, Artificial sequence
  synthetic
PVLELFENGLERLLDALQKKLK

SEQ ID NO: 168 - protein, 22 aa, Artificial sequence
  synthetic
PVLELFEQLLEKLLDALQKKLK

SEQ ID NO: 169 - protein, 22 aa, Artificial sequence
  synthetic
PVLELFENLLEKLLDALQKKLK

SEQ ID NO: 170 - protein, 22 aa, Artificial sequence
  synthetic
  misc_feature: Xaa = Orn
  misc_feature (12)..(12): Xaa can be any naturally occurring amino acid
  misc_feature (19)..(20): Xaa can be any naturally occurring amino acid
  misc_feature (22)..(22): Xaa can be any naturally occurring amino acid
PVLELFENLLEXLLDALQXXLX

SEQ ID NO: 171 - protein, 22 aa, Artificial sequence
  synthetic
PVLELFENLLEKLLDLLQKKLK

SEQ ID NO: 172 - protein, 22 aa, Artificial sequence
  synthetic
PVLELFLNLLERLGDALQKKLK

SEQ ID NO: 173 - protein, 22 aa, Artificial sequence
  synthetic
PVLDLFDNLLDRLLDLLNKKLK

SEQ ID NO: 174 - protein, 22 aa, Artificial sequence
  synthetic
PVLELFENLLERLLDALQKKLK

SEQ ID NO: 175 - protein, 22 aa, Artificial sequence
  synthetic
PVLELFENLLERLLELLNKKLK

SEQ ID NO: 176 - protein, 22 aa, Artificial sequence
  synthetic
PVLELWENLLERLLDALQKKLK

SEQ ID NO: 177 - protein, 22 aa, Artificial sequence
  synthetic
GVLELFLNLLERLLDALQKKLK

SEQ ID NO: 178 - protein, 22 aa, Artificial sequence
  synthetic
PVLELFDNLLEKLLEALQKKLR

SEQ ID NO: 179 - protein, 22 aa, Artificial sequence
  synthetic
PVLELFDNLLERLLDALQKKLK

SEQ ID NO: 180 - protein, 22 aa, Artificial sequence
  synthetic
PVLELFDNLLDKLLDALQKKLR

SEQ ID NO: 181 - protein, 22 aa, Artificial sequence
  synthetic
PVLELFENLLERWLDALQKKLK

SEQ ID NO: 182 - protein, 22 aa, Artificial sequence
  synthetic
PVLELFENLLEKLLEALQKKLK

SEQ ID NO: 183 - protein, 22 aa, Artificial sequence
  synthetic
PLLELFENLLEKLLDALQKKLK

SEQ ID NO: 184 - protein, 22 aa, Artificial sequence
  synthetic
PVLELFLNLLERLLDAWQKKLK

SEQ ID NO: 185 - protein, 22 aa, Artificial sequence
  synthetic
  misc_feature: Xaa = Orn
  misc_feature (19)..(20): Xaa can be any naturally occurring amino acid
  misc_feature (22)..(22): Xaa can be any naturally occurring amino acid
PVLELFENLLERLLDALQXXLX

SEQ ID NO: 186 - protein, 22 aa, Artificial sequence
  synthetic
PVLELFEQLLERLLDALQKKLK

SEQ ID NO: 187 - protein, 22 aa, Artificial sequence
  synthetic
PVLELFENLLERLLDALNKKLK

SEQ ID NO: 188 - protein, 22 aa, Artificial sequence
  synthetic
PVLELFENLLDRLLDALQKKLK

SEQ ID NO: 189 - protein, 22 aa, Artificial sequence
  synthetic
DVLELFENLLERLLDALQKKLK

SEQ ID NO: 190 - protein, 22 aa, Artificial sequence
  synthetic
PVLEFWDNLLDKLLDALQKKLR

SEQ ID NO: 191 - protein, 18 aa, Artificial sequence
  synthetic
PVLDLLRELLEELKQKLK

SEQ ID NO: 192 - protein, 18 aa, Artificial sequence
  synthetic
PVLDLFKELLEELKQKLK

SEQ ID NO: 193 - protein, 18 aa, Artificial sequence
  synthetic
PVLDLFRELLEELKQKLK

SEQ ID NO: 194 - protein, 18 aa, Artificial sequence
  synthetic
PVLELFRELLEELKQKLK

SEQ ID NO: 195 - protein, 18 aa, Artificial sequence
  synthetic
PVLELFKELLEELKQKLK

SEQ ID NO: 196 - protein, 18 aa, Artificial sequence
  synthetic
PVLDLFRELLEELKNKLK

SEQ ID NO: 197 - protein, 18 aa, Artificial sequence
  synthetic
PLLDLFRELLEELKQKLK

SEQ ID NO: 198 - protein, 18 aa, Artificial sequence
  synthetic
GVLDLFRELLEELKQKLK

SEQ ID NO: 199 - protein, 18 aa, Artificial sequence
  synthetic
PVLDLFRELWEELKQKLK

SEQ ID NO: 200 - protein, 18 aa, Artificial sequence
  synthetic
NVLDLFRELLEELKQKLK

SEQ ID NO: 201 - protein, 18 aa, Artificial sequence
  synthetic
PLLDLFKELLEELKQKLK

SEQ ID NO: 202 - protein, 18 aa, Artificial sequence
  synthetic
PALELFKDLLEELRQKLR

SEQ ID NO: 203 - protein, 18 aa, Artificial sequence
  synthetic
AVLDLFRELLEELKQKLK

SEQ ID NO: 204 - protein, 18 aa, Artificial sequence
  synthetic
PVLDFFRELLEELKQKLK

SEQ ID NO: 205 - protein, 18 aa, Artificial sequence
  synthetic
PVLDLFREWLEELKQKLK

SEQ ID NO: 206 - protein, 18 aa, Artificial sequence
  synthetic
PLLELLKELLEELKQKLK

SEQ ID NO: 207 - protein, 18 aa, Artificial sequence
  synthetic
PVLELLKELLEELKQKLK

SEQ ID NO: 208 - protein, 18 aa, Artificial sequence
  synthetic
PALELFKDLLEELRQRLK

SEQ ID NO: 209 - protein, 18 aa, Artificial sequence
  synthetic
PVLDLFRELLNELLQKLK

SEQ ID NO: 210 - protein, 18 aa, Artificial sequence
  synthetic
PVLDLFRELLEELKQKLK

SEQ ID NO: 211 - protein, 18 aa, Artificial sequence
  synthetic
  misc_feature: Xaa = Orn
  misc_feature (14)..(14): Xaa can be any naturally occurring amino acid
  misc_feature (16)..(16): Xaa can be any naturally occurring amino acid
  misc_feature (18)..(18): Xaa can be any naturally occurring amino acid
PVLDLFRELLEELXQXLX

SEQ ID NO: 212 - protein, 18 aa, Artificial sequence
  synthetic
  misc_feature: Xaa = Orn
  misc_feature (7)..(7): Xaa can be any naturally occurring amino acid
  misc_feature (14)..(14): Xaa can be any naturally occurring amino acid
  misc_feature (16)..(16): Xaa can be any naturally occurring amino acid
PVLDLFXELLEELXQXLK

SEQ ID NO: 213 - protein, 18 aa, Artificial sequence
  synthetic
PALELFKDLLEEFRQRLK

SEQ ID NO: 214 - protein, 18 aa, Artificial sequence
  synthetic
PVLDLFRELLEELKQKLK

SEQ ID NO: 215 - protein, 18 aa, Artificial sequence
  synthetic
PVLDLFRELLEEWKQKLK

SEQ ID NO: 216 - protein, 18 aa, Artificial sequence
  synthetic
PVLELFKELLEELKQKLK

SEQ ID NO: 217 - protein, 18 aa, Artificial sequence
  synthetic
PVLDLFRELLELLKQKLK

SEQ ID NO: 218 - protein, 18 aa, Artificial sequence
  synthetic
PVLDLFRELLNELLQKLK

SEQ ID NO: 219 - protein, 18 aa, Artificial sequence
  synthetic
PVLDLFRELLNELWQKLK

SEQ ID NO: 220 - protein, 18 aa, Artificial sequence
  synthetic
PVLDLFRELLEELQKKLK

SEQ ID NO: 221 - protein, 18 aa, Artificial sequence
  synthetic
DVLDLFRELLEELKQKLK

SEQ ID NO: 222 - protein, 18 aa, Artificial sequence
  synthetic
PVLDAFRELLEALLQLKK

SEQ ID NO: 223 - protein, 18 aa, Artificial sequence
  synthetic
PVLDAFRELLEALAQLKK

SEQ ID NO: 224 - protein, 18 aa, Artificial sequence
  synthetic
PVLDLFREGWEELKQKLK

SEQ ID NO: 225 - protein, 18 aa, Artificial sequence
  synthetic
PVLDAFRELAEALAQLKK

SEQ ID NO: 226 - protein, 18 aa, Artificial sequence
  synthetic
PVLDAFRELGEALLQLKK

SEQ ID NO: 227 - protein, 18 aa, Artificial sequence
  synthetic
PVLDLFRELGEELKQKLK

SEQ ID NO: 228 - protein, 18 aa, Artificial sequence
  synthetic
PVLDLFREGLEELKQKLK

SEQ ID NO: 229 - protein, 18 aa, Artificial sequence
  synthetic
PVLDLFRELLEEGKQKLK

SEQ ID NO: 230 - protein, 18 aa, Artificial sequence
  synthetic
PVLELFERLLEDLQKKLK

SEQ ID NO: 231 - protein, 18 aa, Artificial sequence
  synthetic
PVLDLFRELLEKLEQKLK

SEQ ID NO: 232 - protein, 18 aa, Artificial sequence
  synthetic
PLLELFKELLEELKQKLK

SEQ ID NO: 233 - protein, 18 aa, Artificial sequence
  synthetic
LDDLLQKWAEAFNQLLKK

SEQ ID NO: 234 - protein, 18 aa, Artificial sequence
  synthetic
EWLKAFYEKVLEKLKELF

SEQ ID NO: 235 - protein, 18 aa, Artificial sequence
  synthetic
EWLEAFYKKVLEKLKELF

SEQ ID NO: 236 - protein, 18 aa, Artificial sequence
  synthetic
DWLKAFYDKVAEKLKEAF

SEQ ID NO: 237 - protein, 18 aa, Artificial sequence
  synthetic
DWFKAFYDKVFEKFKEFF

SEQ ID NO: 238 - protein, 18 aa, Artificial sequence
  synthetic
GIKKFLGSIWKFIKAFVG

SEQ ID NO: 239 - protein, 18 aa, Artificial sequence
  synthetic
DWFKAFYDKVAEKFKEAF

SEQ ID NO: 240 - protein, 18 aa, Artificial sequence
  synthetic
DWLKAFYDKVAEKLKEAF

SEQ ID NO: 241 - protein, 18 aa, Artificial sequence
  synthetic
DWLKAFYDKVFEKFKEFF

SEQ ID NO: 242 - protein, 18 aa, Artificial sequence
  synthetic
EWLEAFYKKVLEKLKELP

SEQ ID NO: 243 - protein, 18 aa, Artificial sequence
  synthetic
DWFKAFYDKFFEKFKEFF

SEQ ID NO: 244 - protein, 18 aa, Artificial sequence
  synthetic
EWLKAFYEKVLEKLKELF

SEQ ID NO: 245 - protein, 18 aa, Artificial sequence
  synthetic
EWLKAEYEKVEEKLKELF

SEQ ID NO: 246 - protein, 18 aa, Artificial sequence
  synthetic
EWLKAEYEKVLEKLKELF

SEQ ID NO: 247 - protein, 18 aa, Artificial sequence
  synthetic
EWLKAFYKKVLEKLKELF

SEQ ID NO: 248 - protein, 15 aa, Artificial sequence
  synthetic
PVLDLFRELLEQKLK

SEQ ID NO: 249 - protein, 16 aa, Artificial sequence
  synthetic
PVLDLFRELLEELKQK

SEQ ID NO: 250 - protein, 16 aa, Artificial sequence
  synthetic
PVLDLFRELLEKLKQK

SEQ ID NO: 251 - protein, 15 aa, Artificial sequence
  synthetic
PVLDLFRELLEKLQK

SEQ ID NO: 252 - protein, 16 aa, Artificial sequence
  synthetic
PVLDLFRELLEALKQK

SEQ ID NO: 253 - protein, 16 aa, Artificial sequence
  synthetic
PVLDLFENLLERLKQK

SEQ ID NO: 254 - protein, 16 aa, Artificial sequence
  synthetic
PVLDLFRELLNELKQK

SEQ ID NO: 255 - protein, 18 aa, Artificial sequence
  synthetic
DWLKAFYDKVAEKLKEAF

SEQ ID NO: 256 - protein, 18 aa, Artificial sequence
  synthetic
DWLKAFYDKVAEKLKEAF

SEQ ID NO: 257 - protein, 18 aa, Artificial sequence
  synthetic
DWLKAFYDKVAEKLKEAF

SEQ ID NO: 258 - protein, 18 aa, Artificial sequence
  synthetic
DWFKAFYDKVAEKLKEAF

SEQ ID NO: 259 - protein, 18 aa, Artificial sequence
  synthetic
DWLKAFYDKVAEKFKEAF

SEQ ID NO: 260 - protein, 18 aa, Artificial sequence
  synthetic
DWFKAFYDKVAEKFKEAF

SEQ ID NO: 261 - protein, 18 aa, Artificial sequence
  synthetic
DWLKAFYDKVFEKFKEFF

SEQ ID NO: 262 - protein, 18 aa, Artificial sequence
  synthetic
DWLKAFYDKFFEKFKEFF

SEQ ID NO: 263 - protein, 18 aa, Artificial sequence
  synthetic
DWFKAFYDKFFEKFKEFF

SEQ ID NO: 264 - protein, 18 aa, Artificial sequence
  synthetic
DWLKAFYDKVAEKLKEFF

SEQ ID NO: 265 - protein, 18 aa, Artificial sequence
  synthetic
DWLKAFYDKVFEKFKEAF

SEQ ID NO: 266 - protein, 18 aa, Artificial sequence
  synthetic
DWLKAFYDKVFEKLKEFF

SEQ ID NO: 267 - protein, 18 aa, Artificial sequence
  synthetic
DWLKAFYDKVAEKFKEFF

SEQ ID NO: 268 - protein, 18 aa, Artificial sequence
  synthetic
DWLKAFYDKVFEKFKEFF

SEQ ID NO: 269 - protein, 18 aa, Artificial sequence
  synthetic
EWLKLFYEKVLEKFKEAF

SEQ ID NO: 270 - protein, 18 aa, Artificial sequence
  synthetic
EWLKAFYDKVAEKFKEAF

SEQ ID NO: 271 - protein, 18 aa, Artificial sequence
  synthetic
EWLKAFYDKVAEKLKEFF

SEQ ID NO: 272 - protein, 18 aa, Artificial sequence
  synthetic
EWLKAFYDKVFEKFKEAF

SEQ ID NO: 273 - protein, 18 aa, Artificial sequence
  synthetic
EWLKAFYDKVFEKLKEFF

SEQ ID NO: 274 - protein, 18 aa, Artificial sequence
  synthetic
EWLKAFYDKVAEKFKEFF

SEQ ID NO: 275 - protein, 18 aa, Artificial sequence
  synthetic
EWLKAFYDKVFEKFKEFF

SEQ ID NO: 276 - protein, 14 aa, Artificial sequence
  synthetic
AFYDKVAEKLKEAF

SEQ ID NO: 277 - protein, 14 aa, Artificial sequence
  synthetic
AFYDKVAEKFKEAF

SEQ ID NO: 278 - protein, 14 aa, Artificial sequence
  synthetic
AFYDKVAEKFKEAF

SEQ ID NO: 279 - protein, 14 aa, Artificial sequence
  synthetic
AFYDKFFEKFKEFF

SEQ ID NO: 280 - protein, 14 aa, Artificial sequence
  synthetic
AFYDKFFEKFKEFF

SEQ ID NO: 281 - protein, 14 aa, Artificial sequence
  synthetic
AFYDKVAEKFKEAF

SEQ ID NO: 282 - protein, 14 aa, Artificial sequence
  synthetic
AFYDKVAEKLKEFF

SEQ ID NO: 283 - protein, 14 aa, Artificial sequence
  synthetic
AFYDKVFEKFKEAF

SEQ ID NO: 284 - protein, 14 aa, Artificial sequence
  synthetic
AFYDKVFEKLKEFF

SEQ ID NO: 285 - protein, 14 aa, Artificial sequence
  synthetic
AFYDKVAEKFKEFF

SEQ ID NO: 286 - protein, 14 aa, Artificial sequence
  synthetic
KAFYDKVFEKFKEF

SEQ ID NO: 287 - protein, 14 aa, Artificial sequence
  synthetic
LFYEKVLEKFKEAF

SEQ ID NO: 288 - protein, 14 aa, Artificial sequence
  synthetic
AFYDKVAEKFKEAF

SEQ ID NO: 289 - protein, 14 aa, Artificial sequence
  synthetic
AFYDKVAEKLKEFF

SEQ ID NO: 290 - protein, 14 aa, Artificial sequence
  synthetic
AFYDKVFEKFKEAF

SEQ ID NO: 291 - protein, 14 aa, Artificial sequence
  synthetic
AFYDKVFEKLKEFF

SEQ ID NO: 292 - protein, 14 aa, Artificial sequence
  synthetic
AFYDKVAEKFKEFF

SEQ ID NO: 293 - protein, 14 aa, Artificial sequence
  synthetic
AFYDKVFEKFKEFF

SEQ ID NO: 294 - protein, 18 aa, Artificial sequence
  synthetic
DWLKALYDKVAEKLKEAL

SEQ ID NO: 295 - protein, 18 aa, Artificial sequence
  synthetic
DWFKAFYEKVAEKLKEFF

SEQ ID NO: 296 - protein, 18 aa, Artificial sequence
  synthetic
DWFKAFYEKFFEKFKEFF

SEQ ID NO: 297 - protein, 18 aa, Artificial sequence
  synthetic
EWLKALYEKVAEKLKEAL

SEQ ID NO: 298 - protein, 18 aa, Artificial sequence
  synthetic
EWLKAFYEKVAEKLKEAF

SEQ ID NO: 299 - protein, 18 aa, Artificial sequence
  synthetic
EWFKAFYEKVAEKLKEFF

SEQ ID NO: 300 - protein, 18 aa, Artificial sequence
  synthetic
EWLKAFYEKVFEKFKEFF

SEQ ID NO: 301 - protein, 18 aa, Artificial sequence
  synthetic
EWLKAFYEKFFEKFKEFF

SEQ ID NO: 302 - protein, 18 aa, Artificial sequence
  synthetic
EWFKAFYEKFFEKFKEFF

SEQ ID NO: 303 - protein, 18 aa, Artificial sequence
  synthetic
DFLKAWYDKVAEKLKEAW

SEQ ID NO: 304 - protein, 18 aa, Artificial sequence
  synthetic
EFLKAWYEKVAEKLKEAW

SEQ ID NO: 305 - protein, 18 aa, Artificial sequence
  synthetic
DFWKAWYDKVAEKLKEWW

SEQ ID NO: 306 - protein, 18 aa, Artificial sequence
  synthetic
EFWKAWYEKVAEKLKEWW

SEQ ID NO: 307 - protein, 18 aa, Artificial sequence
  synthetic
DKLKAFYDKVFEWAKEAF

SEQ ID NO: 308 - protein, 18 aa, Artificial sequence
  synthetic
DKWKAVYDKFAEAFKEFL

SEQ ID NO: 309 - protein, 18 aa, Artificial sequence
  synthetic
EKLKAFYEKVFEWAKEAF

SEQ ID NO: 310 - protein, 18 aa, Artificial sequence
  synthetic
EKWKAVYEKFAEAFKEFL

SEQ ID NO: 311 - protein, 18 aa, Artificial sequence
  synthetic
DWLKAFVDKFAEKFKEAY

SEQ ID NO: 312 - protein, 18 aa, Artificial sequence
  synthetic
EKWKAVYEKFAEAFKEFL

SEQ ID NO: 313 - protein, 18 aa, Artificial sequence
  synthetic
DWLKAFVYDKVFKLKEFF

SEQ ID NO: 314 - protein, 18 aa, Artificial sequence
  synthetic
EWLKAFVYEKVFKLKEFF

SEQ ID NO: 315 - protein, 18 aa, Artificial sequence
  synthetic
DWLRAFYDKVAEKLKEAF

SEQ ID NO: 316 - protein, 18 aa, Artificial sequence
  synthetic
EWLRAFYEKVAEKLKEAF

SEQ ID NO: 317 - protein, 18 aa, Artificial sequence
  synthetic
DWLKAFYDRVAEKLKEAF

SEQ ID NO: 318 - protein, 18 aa, Artificial sequence
  synthetic
EWLKAFYERVAEKLKEAF

SEQ ID NO: 319 - protein, 18 aa, Artificial sequence
  synthetic
DWLKAFYDKVAERLKEAF

SEQ ID NO: 320 - protein, 18 aa, Artificial sequence
  synthetic
EWLKAFYEKVAERLKEAF

SEQ ID NO: 321 - protein, 18 aa, Artificial sequence
  synthetic
DWLKAFYDKVAEKLREAF

SEQ ID NO: 322 - protein, 18 aa, Artificial sequence
  synthetic
EWLKAFYEKVAEKLREAF

SEQ ID NO: 323 - protein, 18 aa, Artificial sequence
  synthetic
DWLKAFYDRVAERLKEAF

SEQ ID NO: 324 - protein, 18 aa, Artificial sequence
  synthetic
EWLKAFYERVAERLKEAF

SEQ ID NO: 325 - protein, 18 aa, Artificial sequence
  synthetic
DWLRAFYDKVAEKLREAF

SEQ ID NO: 326 - protein, 18 aa, Artificial sequence
  synthetic
EWLRAFYEKVAEKLREAF

SEQ ID NO: 327 - protein, 18 aa, Artificial sequence
  synthetic
DWLRAFYDRVAEKLKEAF

SEQ ID NO: 328 - protein, 18 aa, Artificial sequence
  synthetic
EWLRAFYERVAEKLKEAF

SEQ ID NO: 329 - protein, 18 aa, Artificial sequence
  synthetic
DWLKAFYDKVAERLREAF

SEQ ID NO: 330 - protein, 18 aa, Artificial sequence
  synthetic
EWLKAFYEKVAERLREAF

SEQ ID NO: 331 - protein, 18 aa, Artificial sequence
  synthetic
DWLRAFYDKVAERLKEAF

SEQ ID NO: 332 - protein, 18 aa, Artificial sequence
  synthetic
EWLRAFYEKVAERLKEAF

SEQ ID NO: 333 - protein, 18 aa, Artificial sequence
  synthetic
FAEKFKEAVKDYFAKFWD

SEQ ID NO: 334 - protein, 18 aa, Artificial sequence
  synthetic
DWFKAFYDKVAEKFKEAF

SEQ ID NO: 335 - protein, 18 aa, Artificial sequence
  synthetic
DWLKAFYDKVAEKLKEAF

SEQ ID NO: 336 - protein, 34 aa, Artificial sequence
  synthetic
PALEDLRQGLLPVLESFKVFLSALEEYTKKLNTQ

SEQ ID NO: 337 - DNA, 23 bp, Artificial sequence
  synthetic
gccagtatgcaagggagctcatg

SEQ ID NO: 338 - protein, 25 aa, Artificial sequence
  synthetic
GASTAMGATCANCARGGEGCLCAMG

SEQ ID NO: 339 - DNA, 23 bp, Artificial sequence
  synthetic
gccagtatgcaatggagctcatg

SEQ ID NO: 340 - protein, 25 aa, Artificial sequence
  synthetic
GASTAMGATCANCAMGGEGCLCATG